European Patent Specification EP 3 527 984 B1, published November 8, 2023. Title: Methods, Devices, Kits and Compositions For Detecting Roundworm, Whipworm and Hookworm. Applicant: Idexx Laboratories, Inc. Elsemore, David Allen Geng, Jinming Flynn, Laurie A. Crawford, Michael. The sequence listing filed with the application follows.

SEQUENCE LISTING (38 sequences)

SEQ ID NO: 1 - DNA, 1210 bp, Trichuris vulpis
cattcactgcggttgtaaaagcagtgcagaaatgaggctggtcttccatgcggttatttacctcacattggggttcctcaccgacgccgtaagagaaaaacgtggcaaatgtcctcctgaaccaccgatcgcaggaaacacgatctactgccgcgatgattttgattgtggaggaagacagaagtgctgtacaattgcagaaggacgtggatgcgtgccgccctatggtgaacaacatttcgaagtggtgaaaccgggtcattgcccagctattccagcggttacgggcatggcgaacttctgtaacactgatggcgactgtgatggaccgaaaaaatgttgtctcacatcgcgcggctacgattgcacacatccattacacttcccaatccagccacaacctccagtaggacagtgccctccttcaaagccccgtatcccaggaaaatgggtagacatctgcgctaagcatgccaactgcccagacccagagaagtgttgcgacacggagtatggcaaccgatgtatggatgttggattagtgccaggacaaggagaaagaccaggcaattgcccgaacgaaccacgaataagaggaactaaatacgattgccgacgagacgatgactgcgacggtgtgcagaaatgctgcttcactgttgagggacgtgagtgcgtggaaccaagtagaaaaccactggacaagcccggacattgtccaccaattcccgctgatgtgggctcagccaggtactgcgacactgatcgggattgtgatggaccaagaaaatgctgcctctcttcgcgtggctatgaatgtaaacatccagtacactatcccgatcgagtggagccactagtaggagaatgcccaccatcacgacctcgcattcctgggaaatgggttgacatctgctctaagcatgccaactgcccagacccagagaaatgttgcgacacggagtatggcaaccgatgtatggacgttggattagtgcctggacaaggagaaaaacctgccaactgcccaaaggaaccacgaataagaggaactaagtacgactgtcgacgggacgatgactgcgatgggaaacaaaagtgctgctacacaactgaaggccgcgaatgcgtccatggtatatggccttaaatggttgcttcttcctataataaaagcaaacgaatcaaaaaaaaaaaaaaaaaaaaaaaa

SEQ ID NO: 2 - DNA, 1059 bp, Trichuris vulpis
gtaagagaaaaacgtggcaaatgtcctcctgaaccaccgatcgcaggaaacacgatctactgccgcgatgattttgattgtggaggaagacagaagtgctgtacaattgcagaaggacgtggatgcgtgccgccctatggtgaacaagatttcgaagtggtgaaaccgggtcattgcccagctattccagcggttacgggcatggcgaacttctgtaacactgatggcgactgtgatggaccgaaaaaatgttgtctcacatcgcgcggctacgattgtacacatccgttacacttcccaatccagccacaacctccagtaggacagtgccctccttcaaagccccgtgttccaggaaaatgggtagacatctgcgctaagcatgccaattgcccagacccagagaagtgttgcgacacggagtatggcaaccgatgtatggatgttggattagtggcaggacaaggagaaagaccaggcaattgcccgaacgaaccacgaataagaggaactaaatacgattgccgacgagacgatgactgcgacggtgtgcagaaatgctgcttcactgttgagggacgtgagtgcgtggaaccaagcagaaaaccactggacaagcccggacattgtccaccaattcccgctgatgtgggctcagccaggtactgcgacactgatcgggattgtgatggaccaagaaaatgctgcctctcttcgcgtggctatgaatgtaaacatccagtacactatcccgatcgagtggagccactagtaggagaatgcccaccatcacgacctcgcattcctgggaaatgggttgacatctgctctaagcatgccaactgcccagacccagagaaatgttgcgacacggagtatggcaaccgatgtatggacgttggattagtgcctggacaaggagaaaaacctgccaactgcccaaaggaaccacgaataaggggaactaagtacgactgtcgacgggacgatgactgcgatgggaaacaaaagtgctgctacacaactgaaggccgcgaatgcgtccatggtatatggcct

SEQ ID NO: 3 - protein, 372 aa, Trichuris vulpis
MRLVFHAVIYLTLGFLTDAVREKRGKCPPEPPIAGNTIYCRDDFDCGGRQKCCTIAEGRGCVPPYGEQHFEVVKPGHCPAIPAVTGMANFCNTDGDCDGPKKCCLTSRGYDCTHPLHFPIQPQPPVGQCPPSKPRIPGKWVDICAKHANCPDPEKCCDTEYGNRCMDVGLVPGQGERPGNCPNEPRIRGTKYDCRRDDDCDGVQKCCFTVEGRECVEPSRKPLDKPGHCPPIPADVGSARYCDTDRDCDGPRKCCLSSRGYECKHPVHYPDRVEPLVGECPPSRPRIPGKWVDICSKHANCPDPEKCCDTEYGNRCMDVGLVPGQGEKPANCPKEPRIRGTKYDCRRDDDCDGKQKCCYTTEGRECVHGIWP

SEQ ID NO: 4 - protein, 353 aa, Trichuris vulpis
VREKRGKCPPEPPIAGNTIYCRDDFDCGGRQKCCTIAEGRGCVPPYGEQDFEVVKPGHCPAIPAVTGMANFCNTDGDCDGPKKCCLTSRGYDCTHPLHFPIQPQPPVGQCPPSKPRVPGKWVDICAKHANCPDPEKCCDTEYGNRCMDVGLVAGQGERPGNCPNEPRIRGTKYDCRRDDDCDGVQKCCFTVEGRECVEPSRKPLDKPGHCPPIPADVGSARYCDTDRDCDGPRKCCLSSRGYECKHPVHYPDRVEPLVGECPPSRPRIPGKWVDICSKHANCPDPEKCCDTEYGNRCMDVGLVPGQGEKPANCPKEPRIRGTKYDCRRDDDCDGKQKCCYTTEGRECVHGIWP

SEQ ID NO: 5 - protein, 354 aa, Artificial
  Synthetic
MVREKRGKCPPEPPIAGNTIYCRDDFDCGGRQKCCTIAEGRGCVPPYGEQHFEVVKPGHCPAIPAVTGMANFCNTDGDCDGPKKCCLTSRGYDCTHPLHFPIQPQPPVGQCPPSKPRIPGKWVDICAKHANCPDPEKCCDTEYGNRCMDVGLVPGQGERPGNCPNEPRIRGTKYDCRRDDDCDGVQKCCFTVEGRECVEPSRKPLDKPGHCPPIPADVGSARYCDTDRDCDGPRKCCLSSRGYECKHPVHYPDRVEPLVGECPPSRPRIPGKWVDICSKHANCPDPEKCCDTEYGNRCMDVGLVPGQGEKPANCPKEPRIRGTKYDCRRDDDCDGKQKCCYTTEGRECVHGIWP

SEQ ID NO: 6 - protein, 353 aa, Artificial
  Synthetic
VREKRGKCPPEPPIAGNTIYCRDDFDCGGRQKCCTIAEGRGCVPPYGEQHFEVVKPGHCPAIPAVTGMANFCNTDGDCDGPKKCCLTSRGYDCTHPLHFPIQPQPPVGQCPPSKPRIPGKWVDICAKHANCPDPEKCCDTEYGNRCMDVGLVPGQGERPGNCPNEPRIRGTKYDCRRDDDCDGVQKCCFTVEGRECVEPSRKPLDKPGHCPPIPADVGSARYCDTDRDCDGPRKCCLSSRGYECKHPVHYPDRVEPLVGECPPSRPRIPGKWVDICSKHANCPDPEKCCDTEYGNRCMDVGLVPGQGEKPANCPKEPRIRGTKYDCRRDDDCDGKQKCCYTTEGRECVHGIWP

SEQ ID NO: 7 - protein, 354 aa, Artificial
  Synthetic
MVREKRGKCPPEPPIAGNTIYCRDDFDCGGRQKCCTIAEGRGCVPPYGEQDFEVVKPGHCPAIPAVTGMANFCNTDGDCDGPKKCCLTSRGYDCTHPLHFPIQPQPPVGQCPPSKPRVPGKWVDICAKHANCPDPEKCCDTEYGNRCMDVGLVAGQGERPGNCPNEPRIRGTKYDCRRDDDCDGVQKCCFTVEGRECVEPSRKPLDKPGHCPPIPADVGSARYCDTDRDCDGPRKCCLSSRGYECKHPVHYPDRVEPLVGECPPSRPRIPGKWVDICSKHANCPDPEKCCDTEYGNRCMDVGLVPGQGEKPANCPKEPRIRGTKYDCRRDDDCDGKQKCCYTTEGRECVHGIWP

SEQ ID NO: 8 - protein, 353 aa, Artificial; identical to SEQ ID NO: 4
  Synthetic

SEQ ID NO: 9 - protein, 369 aa, Artificial
  Synthetic
  misc_feature (1)..(19): Xaa can be any naturally occurring amino acid
  misc_feature (69)..(69): Xaa can be any naturally occurring amino acid
  misc_feature (134)..(134): Xaa can be any naturally occurring amino acid
  misc_feature (170)..(170): Xaa can be any naturally occurring amino acid
XXXXXXXXXXXXXXXXXXXVREKRGKCPPEPPIAGNTIYCRDDEDCGGRQKCCTIAEGRGCVPPYGEQXFEVVKPGHCPAIPAVTGMANECNIDGDCDGMCCLISRGYDCTHPLHETIQPQPPVGQCPPSKPRXPGKWVDICAKHANCPDPEKCCDTEYGNRCMDVGLVXGGERPGNCPNEPRIRGIKYDCRRDDDCDGVQKCCETVEGRECVEPSRKPLDKPGHCPPIPADVGSARYCDTDRDCDGPRKCCLSSRGYECKHPVHYPDRVEPLVGECPPSRPRIPGKWVDICSKHANCPDPEKCCDTEYGNRCMDVGLVPGQGEKPANCPKEPRIRGTKYDCRRDDDCDGKQKCCYTTEGRECVHGIWP

SEQ ID NO: 10 - DNA, 865 bp, Toxocara canis
caagaagatttatggtgtggcagcttcgagacgaaggaggcatcacttcacgctcgaaaacagtctggacacccacctgaaatggcttagccacgagcaaaaggaggaactgctgcaaatgaagaaggacggcaaatcgaagaaggagctccaggataagatcatgcactattacgagcacctcgaaggcgatgcgaaacatgaagcaacagagcaactgaagggcggatgccgcgagattcttaagcatgttgttggcgaggagaaagcagctgagatcaaagcactgaaagattctggagcaagcaaagatgagcttaaagccaaggtcgaagaggcactccacgcagtcaccgacgaagaaaagaagcaacatatcgccgaattcggtcccgcatgcaagaagatttatggtgtggcagcttcgagacgaaggaggcatcacttcacgctcgaaaacagtctggacacccacctgaaatggcttagccacgagcaaaaggaggaactgctgcaaatgaagaaggacggcaaatcgaagaaggagctccaggataagatcatgcactattacgagcacctcgaagggatgctcctcgcgctatgtatcctgtattgacggccttccaacctatcacacctgtcagtgcggccttacattcgacgagcgtagaaagacctgtcttcctaagcagctggtaaagtactgcggaatcccagaatctggagaggcgtcggcggaagttggtgagtcgtactaacacagcacgctctcgttggtgcagatgttgtgtgaaatacttttgtcagttttccgtgtgttttaaataaataaaaaattccgtaaaaaaaaaaaaaaaaaaaa

SEQ ID NO: 11 - DNA, 632 bp, Toxocara cati
atttatggtgtggcagcttcgagacgaaggaggcatcacttcacgctcgaaaaaagtctggacacccacctgaaatggcttagccacgagcaaaaggaggaactgctgaaaatgaagaaagatgggaaatcgaagaaggagctccaggataaggtgatgcacttctacgagcacctcgaaggcgatgcgaaacatgaagcaacagagcaactgaagggcggatgccgcgagatccttaagcatgttgttggtgaggagaaagcagctgagatcaaagcactgaaagattctggagcaagcaaagatgagcttaaagccaaggtcgaagatgcactccacgcggtcaccgaagaagaaaagaagcaacatatcgccgaatttggtccagcatgcaaggaaattttcggggtgccggttgatgttcgtcacaaacgcgacccttatactaatatgacgcccgatgaagttgctgaaggactaagaagttaacggtgatcgagctttttgcaaaaactggttgatgcttttaaattcttttaagcctttttcttgtgttatttcggaattgtaccacacgaacagttagttccgaataaagaactgtaattatgtaaaaaaaaaaaaaaaaaaaa

SEQ ID NO: 12 - protein, 205 aa, Toxocara canis
KKIYGVAASRRRRHHFTLENSLDTHLKWLSHEQKEELLQMKKDGKSKKELQDKIMHYYEHLEGDAKHEATEQLKGGCREILKHVVGEEKAAEIKALKDSGASKDELKAKVEEALHAVTDEEKKQHIAEFGPACKKIYGVAASRRRRHHFTLENSLDTHLKWLSHEQKEELLQMKKDGKSKKELQDKIMHYYEHLEGMLLALCILY

SEQ ID NO: 13 - protein, 162 aa, Toxocara cati
IYGVAASRRRRHHFTLEKSLDTHLKWLSHEQKEELLKMKKDGKSKKELQDKVMHFYEHLEGDAKHEATEQLKGGCREILKHVVGEEKAAEIKALKDSGASKDELKAKVEDALHAVTDEEKKQHIAEFGPACKEIFGVPIDVRHKRDPYTNMTPDEVAEGLRS

SEQ ID NO: 14 - protein, 130 aa, Artificial
  Synthetic
MHHFTLENSLDTHLKWLSHEQKEELLQMKKDGKSKKELQDKIMHYYEHLEGDAKHEATEQLKGGCREILKHVVGEEKAAEIKALKDSGASKDELKAKVEEALHAVTDEEKKQHIAEFGPACKKIYGVAAS

SEQ ID NO: 15 - protein, 129 aa, Artificial
  Synthetic
HHFTLENSLDTHLKWLSHEQKEELLQMKKDGKSKKELQDKIMHYYEHLEGDAKHEATEQLKGGCREILKHVVGEEKAAEIKALKDSGASKDELKAKVEEALHAVTDEEKKQHIAEFGPACKKIYGVAAS

SEQ ID NO: 16 - protein, 155 aa, Artificial
  Synthetic
  misc_feature (1)..(11): Xaa can be any naturally occurring amino acid
  misc_feature (18)..(18): Xaa can be any naturally occurring amino acid
  misc_feature (37)..(37): Xaa can be any naturally occurring amino acid
  misc_feature (52)..(52): Xaa can be any naturally occurring amino acid
  misc_feature (55)..(55): Xaa can be any naturally occurring amino acid
  misc_feature (110)..(110): Xaa can be any naturally occurring amino acid
  misc_feature (133)..(133): Xaa can be any naturally occurring amino acid
  misc_feature (135)..(135): Xaa can be any naturally occurring amino acid
  misc_feature (138)..(155): Xaa can be any naturally occurring amino acid
XXXXXXXXXXXHHFTLEXSLDTHLKWLSHEQKEELLXMKKDGKSKKELQDKXMHXYEHLEGDAKHEATEQLKGGCREILKHVVGEEKAAEIFALKDSGASKDELKAKVEXALHAVTDEEKKQHIAEFGFACKXIXGVXXXXXXXXXXXXXXXXXX

SEQ ID NO: 17 - DNA, 535 bp, Toxocara canis
agtcagtagccactttaatccatcagaatgctctctgttcttgcgcttttcgctcttattacttttgctgtggccggtccggaaagctgcggtccaaacgaagtgtggactgaatgtaccggttgcgaattgaaatgtgggcaagatgaaaatacgccgtgcacactaaactgtcgaccgccgtgatgtgagtgctctccaggaagaggcatgagacgaaccaacgatggaaggtgcattccggctagtcagtgcccgcaacacagggccaagagagaggagcaatgcaagccaaatgagcagtggtcaccgtgccgaggatgtgaaggaacatgcgcacaaagatttgtcccttgcactagaaactgccgaccaccaggctgtgaatgcgttgctggcgcaggtttcgtacgtgacgctgaaggaaactgcatcaagttcgacgattgcccgaagtaaataataaccatacaaattgctgattccaattaaaataataaatgagtccagctgttaaaaaaaaaaaaaaaaaaaa

SEQ ID NO: 18 - DNA, 536 bp, Toxocara cati
cagtcagcagctacttttatccatcggaatgctctctgttcttgcgcttttcgctcttattactttcgctgtggccgatccgaaaagttgcggtccaaacgaagtgtggactgaatgtaccggttgcgagttgaaatgcgggcaggatgaggatacgccgtgcacactaaactgtcggccgccgtcatgtgagtgctcaccaggaagaggcatgagacgaaccgacgatgggaggtgcattccggctagtcagtgcccgcaacacagagccaagagagaggagcagtgcaagccaaatgagcagtggtcaccgtgccgaggatgtgaaggaacatgcgcacaaagatttgtcccttgcactagaaactgccgaccaccaggatgtgaatgcgttgctggcgcaggtttcgtacgtgacgctgcaggaaattgcatcaagttcgacgattgcccgaagtaaataataaccatactaattgctgattacaattaaaataataaatgagtccagctgttaaaaaaaaaaaaaaaaaaaa

SEQ ID NO: 19 - protein, 143 aa, Toxocara canis
MLSVLALFALITFAVAGPESCGPNEVWTECTGCELKCGQDENTPCTLNCRPPSCECSPGRGMRRTNDGRCIPASQCPQHRAKREEQCKPNEQWSPCRGCEGTCAQRFVPCTRNCRPPGCECVAGAGFVRDAEGNCIKFDDCPK

SEQ ID NO: 20 - protein, 143 aa, Toxocara cati
MLSVLALFALITFAVADPKSCGPNEVWTECTGCELKCGQDEDTPCTLNCRPPSCECSPGRGMRRTDDGRCIPASQCPQHRAKREEQCKPNEQWSPCRGCEGTCAQRFVPCTRNCRPPGCECVAGAGFVRDAAGNCIKFDDCPK

SEQ ID NO: 21 - protein, 128 aa, Artificial
  Synthetic
MGPESCGPNEVWTECTGCELKCGQDENTPCTLNCRPPSCECSPGRGMRRTNDGRCIPASQCPQHRAKREEQCKPNEQWSPCRGCEGTCAQRFVPCTRNCRPPGCECVAGAGFVRDAEGNCIKFDDCPK

SEQ ID NO: 22 - protein, 127 aa, Artificial
  Synthetic
GPESCGPNEVWTECTGCELKCGQDENTPCTLNCRPPSCECSPGRGMRRTNDGRCIPASQCPQHRAKREEQCKPNEQWSPCRGCEGTCAQRFVPCTRNCRPPGCECVAGAGFVRDAEGNCIKFDDCPK

SEQ ID NO: 23 - protein, 143 aa, Artificial
  Synthetic
  misc_feature (1)..(17): Xaa can be any naturally occurring amino acid
  misc_feature (19)..(19): Xaa can be any naturally occurring amino acid
  misc_feature (42)..(42): Xaa can be any naturally occurring amino acid
  misc_feature (66)..(66): Xaa can be any naturally occurring amino acid
  misc_feature (132)..(132): Xaa can be any naturally occurring amino acid
XXXXXXXXXXXXXXXXXPXSCGPNEVWTECTGCELKCGQDEXTPCTLNCRPPSCECSPGRGMRRTXDGRCIPASQCPQHRAKREEQCKPNEQWSPCRGCEGTCAQRFVPCTRNCRPPGCECVAGAGFVRDAXGNCIKFDDCPK

SEQ ID NO: 24 - DNA, 469 bp, Toxocara canis
atcagcaggtttcgcttcaaatgcttccgataacttttttgctggcaattattgtcggtgcagcagtagctcaccgtaaatgtggtccaaacgaagagtggaccgaatgcactggttgcgaaattaagtgcggtcaaggagagcaaccatgccctatgatgtgtcgtccgccatcgtgtgaatgcatggccggcaaaggattacgaagaacagcggacggaagatgcgtgccggaggcacaatgcccaaaaagaatggtaaagcgagacgaaaaatgtgggccaaacgagaaattcctgaagtgcagaggttgtgagggtacctgcaaagaacgtctcgttccctgccctagaatgtgcaaaccaccaggttgcgaatgccccgcttcagaaggattcgttcgcaatgacaaaggcgaatgtatcaagttcgacgactgcccgaaataaattcaataaatcaattttgt

SEQ ID NO: 25 - DNA, 548 bp, Toxocara cati
atcagcaggtttcgcttcaaatgcttccgttaacttttttgctggcatttattgtgggtgcagcggtagctcaccgtaaatgtggtccaaatgaagagtggacggaatgcactggctgcgaaatgaagtgcggtgaaggagagacaccatgccctatgatgtgtcgtccgccatcgtgtgaatgcatggccggcaaaggattacgaagaacaccggacggaagatgtgtgccggaggcacaatgcccgaaacatatggtaaagcgagatgaaaaatgtgggaaaaacgagaaattcctgaagtgcagaggatgtgagggtacgtgcaaagaacgtctcgtgccgtgccctaagatgtgcaaaccaccaggttgcgaatgcccggcttcggaaggattcgttcgcaatgacaaacacgaatgtatcaagttcgacgactgccccaaataaattcaataaatcagtcttgttgataaatacaatcgtgatgctcacgtttttttttcttgccataaaatctatacttcccaaaaaaaaaaaaaaaaaaaa

SEQ ID NO: 26 - protein, 142 aa, Toxocara canis
MLPITFLLAIIVGAAVAHRKCGPNEEWTECTGCEIKCGQGEQPCPMMCRPPSCECMAGKGLRRTADGRCVPEAQCPKRMVKRDEKCGPNEKFLKCRGCEGTCKERLVPCPRMCKPPGCECPASEGFVRNDKGECIKFDDCPK

SEQ ID NO: 27 - protein, 142 aa, Toxocara cati
MLPLTFLLAFIVGAAVAHRKCGPNEEWTECTGCEMKCGEGETPCPMMCRPPSCECMAGKGLRRTPDGRCVPEAQCPKHMVKRDEKCGKNEKFLKCRGCEGTCKERLVPCPKMCKPPGCECPASEGFVRNDKHECIKFDDCPK

SEQ ID NO: 28 - protein, 126 aa, Artificial
  Synthetic
MHRKCGPNEEWTECTGCEIKCGQGEQPCPMMCRPPSCECMAGKGLRRTADGRCVPEAQCPKRMVKRDEKCGPNEKFLKCRGCEGTCKERLVPCPRMCKPPGCECPASEGFVRNDKGECIKFDDCPK

SEQ ID NO: 29 - protein, 125 aa, Artificial
  Synthetic
HRKCGPNEEWTECTGCEIKCGQGEQPCPMMCRPPSCECMAGKGLRRTADGRCVPEAQCPKRMVKRDEKCGPNEKFLKCRGCEGTCKERLVPCPRMCKPPGCECPASEGFVRNDKGECIKFDDCPK

SEQ ID NO: 30 - protein, 142 aa, Artificial
  Synthetic
  misc_feature (1)..(17): Xaa can be any naturally occurring amino acid
  misc_feature (35)..(35): Xaa can be any naturally occurring amino acid
  misc_feature (39)..(39): Xaa can be any naturally occurring amino acid
  misc_feature (42)..(42): Xaa can be any naturally occurring amino acid
  misc_feature (65)..(65): Xaa can be any naturally occurring amino acid
  misc_feature (78)..(78): Xaa can be any naturally occurring amino acid
  misc_feature (88)..(88): Xaa can be any naturally occurring amino acid
  misc_feature (111)..(111): Xaa can be any naturally occurring amino acid
  misc_feature (132)..(132): Xaa can be any naturally occurring amino acid
XXXXXXXXXXXXXXXXXHRKCGPNEEWTECTGCEXKCGXGEXPCPMMCRPPSCECMAGKGLRRTXDGRCVPEAQCPKXMVKRDEKCGXNEKFLKCRGCEGTCKERLVPCPXMCKPPGCECPASEGFVRNDKXECIKFDDCPK

SEQ ID NO: 31 - DNA, 1343 bp, Ancylostoma
atgggcagcagccatcatcatcatcatcacagcagcggcctggtgccgcgcggcagccatatggctagcatgactggtggacagcaaatgggtcgcggatccgaattcgagctcaccacttgtccaggaaatgatctaacagatgctgaacgcacactgctaactagggtgcacaattccattcgacgggaaatagcgcaaggagttgcaaacaactaccatggtggtaaactgcctgctggaaagaacatatacaggatgagatacagctgtgagctggaacaggctgctattgatgctagtcaaaccttctgttccgcatcattggaggaaccacagaaatatggacaaaacatccaagcatacgtcacaccatctataatcgctcgcccgaaaaacgaccttcttgaagatgcagtgaaacaatggtatctgcctgttatctactacggccaacgcgacgcggccaacaagttcaccgatccgcgcttgtacacatttgcaaacctcgcctacgacaagaacactgcacttggctgtcactatgcgaaatgtcaaggccctgacagaatcgtcattagttgcatgtacaacaacgtcgttcctgacaacgctgtgatctacgagccaggaactgcttgcgtaaaagatcaggactgcactacttatcctcagtccacatgcaaggacagcctttgcattattcctacgccacatccaccaaatccaccaaatccaccacctgcaatgtgtccaaacgctgaaatgactgatgcagcacgaaagaaggtcctcgacatgcacaactggcgcagatcgcagctcgctctgggaaacgttcaaaacgggaaaaatgcttacaactgccccactgcaacagacatgtacaagatggaatatgattgcgacctcgagaacagcgctctagcgtatgcaaagcaatgtagtctcgttggttcagcagaaggaactcgtccaggagaaggcgagaatgtccacaaaggcgctctcgtaaccgatccggaggctgcagttcagaccgcagttcaagcatggtggagtcaaatctcacaaaatggactcaatgcacagatgaaattcactgctttcttgaaggacaagcctgacgctccgacagcgtttacacagatggcgtgggccaaatccgtaaagcttggatgtgctgtctctaattgtcaggcagataccttcaccgtctgtagatacaaagctgccggaaacatcgtgggcgaattcatctataccaagggaaatgtatgcgacgcctgtaaagccacatgcattaccgcggaaggtctttgcccaacgccttgagcggccgc

SEQ ID NO: 32 - DNA, 767 bp, Ancylostoma
atgggcagcagccatcatcatcatcatcacagcagcggcctggtgccgcgcggcagccatatggctagcatgactggtggacagcaaatgggtcgcggatccgaattcgagctcaccacttgtccaggaaatgatctaacagatgctgaacgcacactgctaactagggtgcacaattccattcgacgggaaatagcgcaaggagttgcaaacaactaccatggtggtaaactgcctgctggaaagaacatatacaggatgagatacagctgtgagctggaacaggctgctattgatgctagtcaaaccttctgttccgcatcattggaggaaccacagaaatatggacaaaacatccaagcatacgtcacaccatctataatcgctcgcccgaaaaacgaccttcttgaagatgcagtgaaacaatggtatctgcctgttatctactacggccagcgcgacgcggccaacaagtttacggatccgcgcttgtacacatttgcaaacctcgcctacgacaagaacactgcacttggctgtcactatgcgaaatgtcaaggccctgacagaatcgtcattagttgcatgtacaacaacgtcgttcctgacaacgcagtgatctacgagcctggaactgcttgcgtaaaagatgcggactgcactacttatcctcagtccacatgcaaggacagcctttgcattattcctacgccacatccaccaaatccaccaaatccaccaccagcaatgagtccatgagcggccgc

SEQ ID NO: 33 - protein, 444 aa, Ancylostoma
MGSSHHHHHHSSGLVPRGSHMASMTGGQQMGRGSEFELTTCPGNDLTDAERTLLTRVHNSIRREIAQGVANNYHGGKLPAGKNIYRMRYSCELEQAAIDASQTFCSASLEEPQKYGQNIQAYVTPSIIARPKNDLLEDAVKQWYLPVIYYGQRDAANKFTDPRLYTFANLAYDKNTALGCHYAKCQGPDRIVISCMYNNVVPDNAVIYEPGTACVKDQDCTTYPQSTCKDSLCIIPTPHPPNPPNPPPAMCPNAEMTDAARKKVLDMHNWRRSQLALGNVQNGKNAYNCPTATDMYKMEYDCDLENSALAYAKQCSLVGSAEGTRPGEGENVHKGALVTDPEAAVQTAVQAWWSQISQNGLNAQMKFTAFLKDKPDAPTAFTQMAWAKSVKLGCAVSNCQADTFTVCRYKAAGNIVGEFIYTKGNVCDACKATCITAEGLCPTP

SEQ ID NO: 34 - protein, 252 aa, Ancylostoma
MGSSHHHHHHSSGLVPRGSHMASMTGGQQMGRGSEFELTTCPGNDLTDAERTLLTRVHNSIRREIAQGVANNYHGGKLPAGKNIYRMRYSCELEQAAIDASQTFCSASLEEPQKYGQNIQAYVTPSIIARPKNDLLEDAVKQWYLPVIYYGQRDAANKFTDPRLYTFANLAYDKNTALGCHYAKCQGPDRIVISCMYNNVVPDNAVIYEPGTACVKDADCTTYPQSTCKDSLCIIPTPHPPNPPNPPPAMSP

SEQ ID NO: 35 - protein, 8 aa, Artificial
  Synthetic
RFVPCTRN

SEQ ID NO: 36 - protein, 10 aa, Artificial
  Synthetic
RDAEGNCIKF

SEQ ID NO: 37 - protein, 64 aa, Artificial
  Synthetic
MGPESCGPNEVWTECTGCELKCGQDENTPCTLNCRPPSCECSPGRGMRRTNDGRCIPASQCPQH

SEQ ID NO: 38 - protein, 65 aa, Artificial
  Synthetic
MRAKREEQCKPNEQWSPCRGCEGTCAQRFVPCTRNCRPPGCECVAGAGFVRDAEGNCIKFDDCPK